European Patent Application EP 4 582 537 A1, published July 9, 2025. Title: Proteins, polynucleotides, expression vectors, transformants, plasmalogen-containing compositions, and a method for producing plasmalogen. Applicant: INSTITUTE OF RHEOLOGICAL FUNCTION OF FOOD CO., LTD. The sequence listing filed with the application follows.

SEQUENCE LISTING (4 sequences)

SEQ ID NO: 1 - protein, 1416 aa, Enterococcus faecalis
MMVMRAGIDVGSTTVKLVFLNKQNQPIFTKYERHFSDVKAATERILKEGLARIGADQPVTMSITGSGGMGLAEVLGIPFVQEVIACTRTVETIIPETDVAIELGGEDAKITFFDGALEQRMNGSCAGGTGAFIDQMAVLLKTDANGVNELAKNYQTIYPIASRCGVFAKTDVQPLINEGAAKEDIAASIFQAVVNQTIAGLAAGRKIKGKVAFLGGPLFFMSELRKRFVETLAIQTEDVIFPEQPQLFVAMGAALYSEDAAECTLEELIQRLVNSQATDLQPSDTLPPLFNSAEDLADFRERHAQAQATEKPLSQHTGVTFLGIDAGSTTTKVTLIDEDGHLLFSFYGNNQGQPLETTMTVLKSLYQQLPEEVFIGKAAVTGYGEQLIKNALKVDIGEVETMAHYKAANHFQPGVDFILDIGGQDMKAMTIKNGVLSSIQLNEACSSGCGSFIETFAQSLKYNVKDFALAALESQAPVDLGSRCTVFMNSKVKQVQKEGASVGDISAGLSYSVIKNAIYKVIKVRRPEELGEKIVCQGGTFYNEAVLRAFEKISGREVVRPSIAGLMGAYGAALIALDAYEIGEETTLLSLEELAAFTSEKEFTHCGLCENNCQLTVTVFSDGRQFITGNRCERGARIKIKREERKVNLVDYKYRKLFKYRPLRENKAFRGRLGIPRVLNMYENYPLWHTFFTDLGFRVELSPRSNKQIYEQGLETIPSDTVCYPAKMAHGHIQALIDAQVPIIFYPGVVFEQQETVEADNHFNCPIVQSYPDVIRNNVDAIREGQVDYRNPYLNLANEAAVAKVLAENFADLGISLEEIQTALHHGYQELAAFKKEIQEKGEETLAMLTEKGQRGIVLSGRPYHLDPEINHGIAEVITQEGFHVLTEDSISHLGDVQNLRVVNQWVYHSRLYAAAKVVAKTKNLELVQLNSFGCGLDAVTTDQVEEIMDRSGKIYTVLKIDEGANLGAIRIRLRSLKAAVNEREKQQFVPHMQMEEPEKIVFTKQMKKTHTLLLPMLSPIHQSGLVDVALQASGYHVVCLPAQDKEAVNVGLKYVNNDACYPAIISIGQLVEALESGQYDLDNVSVLMTQTGGGCRATNYIPLLRKALNDAGFSQVPVVSVSMGNKGVESNPGFKFTLPMIKRLVVAFLYGDLFERVVYRTRPYETEKGMVDQLHQDWLKRVEANVRNGSLTQFNHFMKKIIRTFDEIPLQEIKKPKVGVVGEILVKYSPTANNDIVRLLEEEGAEAVVPDIVGFMNYSLYNQIWKYENMGMSKQSKRLAEFAIKIIELVEKPMDKALRKSVRFDGIHSIYDMAADASKILSIGNHTGEGWFLTAEMIELLKHEVNNIVCMQPFGCLPNHIVGKGVVKELRRQYPQANIAAVDYDPGVSLVNQLNRIRLMMATANKLLKEENVKR

SEQ ID NO: 2 - protein, 1639 aa, Bifidobacterium longum
MVDIVTDASVKPASHPKPLRVGLDIGSTTVKAVVLDQTDSLDAVLFSDYRRHHANVRATVAGLLEDIHKELESRGRGDEPIRLAITGSGGLALADNLHVPFVQEVIAETEAIDKEYPQADVIIELGGEDAKITYLKPTPEQRMNGSCAGGTGAFIDQMSTLLDTDAAGLNEMAKSYENLYPIASRCGVFAKTDLQPLINDGAAKPDLAASIFTAVATQTIAGLAAGRPIHGTVIFLGGPLFFMSELRAAFQRALEGKVDEFIVPTDAHLYVAYGSALQADMDSDDQGHHFEAHTCDEILMRLDELKNLPSNTPTMPPLFPTEADREDFNKRHHKEHIHIGTLEGAHGPHFLGIDAGSTTIKATLVNDDREIVWSSYANNEGSPLTAAINIVKKIQSELPEGAWIARSCATGYGEGLITTGLHLDEGVVETMAHYRGAEMVSPGVTAVIDIGGQDMKYLAITDGVIDSIAVNEACSSGCGSFLQTFAMSMGLTIQEFTQKALASTHPVDLGSRCTVFMNSSVKQAQKEGASIEDIAAGLCYSVVRNALYKVIKLRDSGELGDTVVVQGGTFLNDAVLRAFELLTERQVTRPNIAGLMGAFGAALTARMHYQDEADHLDVVVKADGSEEQSEAEPAPKSEPKAAAFKKTETAKPEVHVVVVDGVTHTASSILTGEALDNMSMTTERDVCKLCQNHCKLTITTFSDGSRFVTGNRCERGGDAKKKRSDRPNLYDYKYKRCFAYRRLTDKKATRGEIGIPRALNMYENYPFWFTLLTTLGFKVMISGRSSHELFETGIESIASENICYPAKLVHGHIKWLLNKGIKTIFYPCVSYEENLVPNTDNHYNCPVVANYPLVVGANMPELREDGVRYMHPYFNLANHELMVDRILEEFAWADVTREEVETAVKAAYAEDKVFKHDVQQEGLTALAYMKEHNCRGIVLAGRPYHIDPEINHGIPETICSLGMVVLSEDSICELQPGEKLNLTEFLSEGEADPRSKNAAGFRHVGDRTVTKMPLRVTNQWAYHSRLYAAAHFVASYPGLELVQLNSFGCGLDAITTDQVAEILADKADVYTLLKIDEVSNLGAAKIRLRSLKAAVEEREANKAREAAAAKAVQGPKSAGFRKTGSTAPTPGRQILLDSTMAANPKLTKAMRAASKRAAERDLQAAVASKNGTSDGTTGVTNAKNAKKSGHNNATMSRYAHREKFVKDMKKNYTIVGPQMSPIHMSLVEAVIRSGGYKFDILKHASRGDVETGLKYVNNDACYPAIMVIGQLIDAILEGEYDPDHVALAITQTGGMCRATNYFGLIRKALVDAGYPQIPVIAISTQGLEDNPGFKATLPLLHRAIKALILGDLLMKCLYRVRPYEVEKGSANKLYELWDTIVRETIEHHGYSKTAAKAPSIKKGYLPYNVLAKEIVKSFDNLPLRDIPRKVRVGVVGEILVKYQPDANNHVVDVIESQDCEAVVPGIMEFMTTRPYITDWNEKNLGMGGNKTVYALMRKGLDLYNAPIKAALATSNGKFKQDEPMPELVKKAAEVTSIGVQAGEGWLLTAEILELIEQGCPNVICAQPFACLPNHVTGRGMFGKIRRLHPEANIVSIDYDPGASEANQLNRIKLMIAAAKKAHNAKFAEAGEPQGFTSAD

SEQ ID NO: 3 - DNA, 39 bp, synthetic construct
  source 1..39: mol_type = other DNA
cgcgaacagattggaggtgttatgagagcagggattgat

SEQ ID NO: 4 - DNA, 39 bp, synthetic construct
  source 1..39: mol_type = other DNA
gtggcggccgctctattatctttttacattttcttcttt